European Patent Application EP 4 438 048 A1, published October 2, 2024. Title: Pharmaceutical composition for the treatment or prevention of T-cell related diseases. Applicant: RegCell Co., Ltd. Application JP. The sequence listing filed with the application follows.

SEQUENCE LISTING (2 sequences)

SEQ ID NO: 1 - DNA, 25 bp, synthetic construct
  misc_feature 1..25: note = Forward primer used in Example
  source 1..25: mol_type = other DNA
ttgggttaagtttgttgtaggatag

SEQ ID NO: 2 - DNA, 25 bp, synthetic construct
  misc_feature 1..25: note = Reverse primer used in Example
  source 1..25: mol_type = other DNA
atctaaaccctattatcacaacccc